European Patent Application EP 4 491 634 A1, published January 15, 2025. Title: Anti-Trop2 antibodies in immunosuppressed subjects. Applicant: ADRIATX S.r.l. The sequence listing filed with the application follows.

SEQUENCE LISTING (5 sequences)

SEQ ID NO: 1 - DNA, 328 bp, synthetic construct
  source 1..328: mol_type = other DNA
cagctgcagcagtctggagctgaggtggtgaagcgtggggcttcagtgaagctgtcctgcaagacttctggcttcaccttcagcagtagctatataagttggttgaagcagaagcctcgacagagtcttgagtggattgcatggattatgctggaactggtggtactagctataatcagaagttcacaggcaaggcccaactgactgtagacacatcctccagcacagcctacatgcaactcagcagcctgacatctgaggactctgccatctattactgtgcaagacataacccttgttactatgctatggattactggggtcaagg

SEQ ID NO: 2 - protein, 109 aa, synthetic construct
DVQLEQFGAELVRPGTSVKMSCKAAGYTFTNYWIGWVKQRPGHGLEWIGDIYPGGGYTNYNEKFKGKATLTADTSSSTAYMQLSSLTFEDFAIYYCARGTGGGDYWGQG

SEQ ID NO: 3 - DNA, 381 bp, synthetic construct
  source 1..381: mol_type = other DNA
atgttctcactagctcttctcctcagtcttcttctcctctgtgtctctgattctagggcagaaacaactgtgacccagtctccagcatccctgtccatggctataggagaaaaagtctccatcagatgcataaccagcactgatattgatgatgatatgaactggtaccagcagaagccaggggaacctcctaagctccttatttcagaaggcaatactcttcgtcctggagtcccatcccgattctccagcagtggctatggtacagattttgtttttacaattgaaaacatgctctcagaagatgttgcagattactactgtttgcaaagtgataacttgccgtacacgttcggaggggggaccaagctggaaataaaa

SEQ ID NO: 4 - protein, 127 aa, synthetic construct
MFSLALLLSLLLLCVSDSRAETTVTQSPASLSMAIGEKVSIRCITSTDIDDDMNWYQQKPGEPPKLLISEGNTLRPGVPSRFSSSGYGTDFVFTIENMLSEDVADYYCLQSDNLPYTFGGGTKLEIK

SEQ ID NO: 5 - protein, 127 aa, synthetic construct
MFSLALLLSLLLLCVSDSRAETTVTQSPASLSMAIGEKVTIRCITSTDIDDDMNWYQQKPGEPPKLLISEGNTLRPGVPSRFSSSGYGTDFVFTIENMLSEDVADYYCLQSDNLPYTFGGGTKLEIK